European Patent Application EP 4 663 759 A1, published December 17, 2025. Title: 生物酶突变体及其制备方法和应用. Applicant: 上海联影微电子科技有限公司. The sequence listing filed with the application follows.

SEQUENCE LISTING (88 sequences)

SEQ ID NO: 1 - protein, 605 aa, synthetic construct
MQTLLVSSLVVSLAAALPHYIRSNGIEASLLTDPKDVSGRTVDYIIAGGGLTGLTTAARLTENPNISVLVIESGSYESDRGPIIEDLNAYGDIFGSSVDHAYETVELATNNQTALIRSGNGLGGSTLVNGGTWTRPHKAQVDSWETVFGNEGWNWDNVAAYSLQAERARAPNAKQIAAGHYFNASCHGVNGTVHAGPRDTGDDYSPIVKALMSAVEDRGVPTKKDFGCGDPHGVSMFPNTLHEDQVRSDAAREWLLPNYQRPNLQVLTGQYVGKVLLSQNGTTPRAVGVEFGTHKGNTHNVYAKHEVLLAAGSAVSPTILEYSGIGMKSILEPLGIDTVVDLPVGLNLQDQTTATVRSRITSAGAGQGQAAWFATFNETFGDYSEKAHELLNTKLEQWAEEAVARGGFHNTTALLIQYENYRDWIVNHNVAYSELFLDTAGVASFDVWDLLPFTRGYVHILDKDPYLHHFAYDPQYFLNELDLLGQAAATQLARNISNSGAMQTYFAGETIPGDNLAYDADLSAWTEYIPYHFRPNYHGVGTCSMMPKEMGGVVDNAARVYGVQGLRVIDGSIPPTQMSSHVMTVFYAMALKISDAILEDYASMQ

SEQ ID NO: 2 - protein, 527 aa, synthetic construct
MADSRDPASDQMQHWKEQRAAQKADVLTTGAGNPVGDKLNVITVGPRGPLLVQDVVFTDEMAHFDRERIPERVVHAKGAGAFGYFEVTHDITKYSKAKVFEHIGKKTPIAVRFSTVAGESGSADTVRDPRGFAVKFYTEDGNWDLVGNNTPIFFIRDPILFPSFIHSQKRNPQTHLKDPDMVWDFWSLRPESLHQVSFLFSDRGIPDGHRHMNGYGSHTFKLVNANGEAVYCKFHYKTDQGIKNLSVEDAARLSQEDPDYGIRDLFNAIATGKYPSWTFYIQVMTFNQAETFPFNPFDLTKVWPHKDYPLIPVGKLVLNRNPVNYFAEVEQIAFDPSNMPPGIEASPDKMLQGRLFAYPDTHRHRLGPNYLHIPVNCPYRARVANYQRDGPMCMQDNQGGAPNYYPNSFGAPEQQPSALEHSIQYSGEVRRFNTANDDNVTQVRAFYVNVLNEEQRKRLCENIAGHLKDAQIFIQKKAVKNFTEVHPDYGSHIQALLDKYNAEKPKNAIHTFVQSGSHLAAREKANL

SEQ ID NO: 3 - protein, 605 aa, synthetic construct
MQTLLVSSLVVSLAAALPHYIRSNGIEASLLTDPKDVSGRTVDYIIAGGGLTGLTTAARLTENPQISVLVIESGSYESDRGPIIEDLNAYGDIFGSSVDHAYETVELATNQQTALIRSGNGLGGSTLVNGGTWTRPHKAQVDSWETVFGNEGWNWDNVAAYSLQAERARAPNAKQIAAGHYFQASCHGVQGTVHAGPRDTGDDYSPIVKALMSAVEDRGVPTKKDFGCGDPHGVSMFPNTLHEDQVRSDAAREWLLPNYQRPNLQVLTGQYVGKVLLSQQGTTPRAVGVEFGTHKGNTHNVYAKHEVLLAAGSAVSPTILEYSGIGMKSILEPLGIDTVVDLPVGLNLQDQTTATVRSRITSAGAGQGQAAWFATFQETFGDYSEKAHELLNTKLEQWAEEAVARGGFHQTTALLIQYENYRDWIVNHNVAYSELFLDTAGVASFDVWDLLPFTRGYVHILDKDPYLHHFAYDPQYFLNELDLLGQAAATQLARQISNSGAMQTYFAGETIPGDNLAYDADLSAWTEYIPYHFRPNYHGVGTCSMMPKEMGGVVDNAARVYGVQGLRVIDGSIPPTQMSSHVMTVFYAMALKISDAILEDYASMQ

SEQ ID NO: 4 - protein, 605 aa, synthetic construct
MQTLLVSSLVVSLAAALPHYIRSNGIEASLLTDPKDVSGRTVDYIIAGGGLTGLTTAARLTENPAISVLVIESGSYESDRGPIIEDLNAYGDIFGSSVDHAYETVELATNAQTALIRSGNGLGGSTLVNGGTWTRPHKAQVDSWETVFGNEGWNWDNVAAYSLQAERARAPNAKQIAAGHYFAASCHGVAGTVHAGPRDTGDDYSPIVKALMSAVEDRGVPTKKDFGCGDPHGVSMFPNTLHEDQVRSDAAREWLLPNYQRPNLQVLTGQYVGKVLLSQAGTTPRAVGVEFGTHKGNTHNVYAKHEVLLAAGSAVSPTILEYSGIGMKSILEPLGIDTVVDLPVGLNLQDQTTATVRSRITSAGAGQGQAAWFATFAETFGDYSEKAHELLNTKLEQWAEEAVARGGFHATTALLIQYENYRDWIVNHNVAYSELFLDTAGVASFDVWDLLPFTRGYVHILDKDPYLHHFAYDPQYFLNELDLLGQAAATQLARAISNSGAMQTYFAGETIPGDNLAYDADLSAWTEYIPYHFRPNYHGVGTCSMMPKEMGGVVDNAARVYGVQGLRVIDGSIPPTQMSSHVMTVFYAMALKISDAILEDYASMQ

SEQ ID NO: 5 - protein, 527 aa, synthetic construct
MADSRDPASDQMQHWKEQRAAQKADVLTTGAGNPVGDKLNVITVGPRGPLLVQDVVFTDEMAHFDRERIPERVVHAKGAGAFGYFEVTHDITKYSKAKVFEHIGKKTPIAVRFSTVAGESGSADTVRDPRGFAVKFYTEDGNWDLVGQNTPIFFIRDPILFPSFIHSQKRNPQTHLKDPDMVWDFWSLRPESLHQVSFLFSDRGIPDGHRHMNGYGSHTFKLVNANGEAVYCKFHYKTDQGIKQLSVEDAARLSQEDPDYGIRDLFNAIATGKYPSWTFYIQVMTFNQAETFPFNPFDLTKVWPHKDYPLIPVGKLVLNRNPVNYFAEVEQIAFDPSNMPPGIEASPDKMLQGRLFAYPDTHRHRLGPNYLHIPVNCPYRARVANYQRDGPMCMQDNQGGAPNYYPNSFGAPEQQPSALEHSIQYSGEVRRFNTANDDQVTQVRAFYVNVLNEEQRKRLCENIAGHLKDAQIFIQKKAVKQFTEVHPDYGSHIQALLDKYNAEKPKNAIHTFVQSGSHLAAREKANL

SEQ ID NO: 6 - DNA, 1743 bp, synthetic construct
  source 1..1743: mol_type = other DNA
atgcagactctccttgtgagctcgcttgtggtctccctcgctgcggccctgccacactacatcaggagcaatggcattgaagccagcctcctgactgatcccaaggatgtctccggccgcacggtcgactacatcatcgctggtggaggtctgactggactcaccaccgctgctcgtctgacggagaacccccaaatcagtgtgctcgtcatcgaaagtggctcctacgagtcggacagaggtcctatcattgaggacctgaacgcctacggcgacatctttggcagcagtgtagaccacgcctacgagaccgtggagctcgctaccaaccaacaaaccgcgctgatccgctccggaaatggtctcggtggctctactctagtgaatggtggcacctggactcgcccccacaaggcacaggttgactcttgggagactgtctttggaaatgagggctggaactgggacaatgtggccgcctactccctccaggctgagcgtgctcgcgcaccaaatgccaaacagatcgctgctggccactacttccaagcatcctgccatggtgttcaaggtactgtccatgccggaccccgcgacaccggcgatgactattctcccatcgtcaaggctctcatgagcgctgtcgaagaccggggcgttcccaccaagaaagacttcggatgcggtgacccccatggtgtgtccatgttccccaacaccttgcacgaagaccaatatgttggtaaggtgctccttagccagcaaggcaccacccctcgtgccgttggcgtggaattcggcacccacaagggcaacacccacaacgtttacgctaagcacgaggtcctcctggccgcgggctccgctgtctctcccacaatcctcgaatattccggtatcggaatgaagtccatcctggagccccttggtatcgacaccgtcgttgacctgcccgtcggcttgaacctgcaggaccagaccaccgctaccgtccgctcccgcatcacctctgctggtgcaggacagggacaggccgcttggttcgccaccttccaagagacctttggtgactattccgaaaaggcacacgagctgctcaacaccaagctggagcagtgggccgaagaggccgtcgcccgtggcggattccaccaaaccaccgccttgctcatccagtacgagaactaccgcgactggattgtcaaccacaacgtcgcgtactcggaactcttcctcgacactgccggagtagccagcttcgatgtgtgggaccttctgcccttcacccgaggatacgttcacatcctcgacaaggacccctaccttcaccacttcgcctacgaccctcagtacttcctcaacgagctggacctgctcggtcaggctgccgctactcaactggcccgccaaatctccaactccggtgccatgcagacctacttcgctggggagactatccccggtgataacctcgcgtatgatgccgatttgagcgcctggactgagtacatcccgtaccacttccgtcctaactaccatggcgtgggtacttgctccatgatgccgaaggagatgggcggtgttgttgataatgctgcccgtgtgtatggtgtgcagggactgcgtgtcattgatggttctattcctcctacgcaaatgtcgtcccatgtcatgacggtgttctatgccatggcgctaaaaatttcggatgctatcttggaagattatgcttccatgcagtga

SEQ ID NO: 7 - DNA, 1743 bp, synthetic construct
  source 1..1743: mol_type = other DNA
atgcagactctccttgtgagctcgcttgtggtctccctcgctgcggccctgccacactacatcaggagcaatggcattgaagccagcctcctgactgatcccaaggatgtctccggccgcacggtcgactacatcatcgctggtggaggtctgactggactcaccaccgctgctcgtctgacggagaaccccgccatcagtgtgctcgtcatcgaaagtggctcctacgagtcggacagaggtcctatcattgaggacctgaacgcctacggcgacatctttggcagcagtgtagaccacgcctacgagaccgtggagctcgctaccaacgcccaaaccgcgctgatccgctccggaaatggtctcggtggctctactctagtgaatggtggcacctggactcgcccccacaaggcacaggttgactcttgggagactgtctttggaaatgagggctggaactgggacaatgtggccgcctactccctccaggctgagcgtgctcgcgcaccaaatgccaaacagatcgctgctggccactacttcgccgcatcctgccatggtgttgccggtactgtccatgccggaccccgcgacaccggcgatgactattctcccatcgtcaaggctctcatgagcgctgtcgaagaccggggcgttcccaccaagaaagacttcggatgcggtgacccccatggtgtgtccatgttccccaacaccttgcacgaagaccaatatgttggtaaggtgctccttagccaggccggcaccacccctcgtgccgttggcgtggaattcggcacccacaagggcaacacccacaacgtttacgctaagcacgaggtcctcctggccgcgggctccgctgtctctcccacaatcctcgaatattccggtatcggaatgaagtccatcctggagccccttggtatcgacaccgtcgttgacctgcccgtcggcttgaacctgcaggaccagaccaccgctaccgtccgctcccgcatcacctctgctggtgcaggacagggacaggccgcttggttcgccaccttcgccgagacctttggtgactattccgaaaaggcacacgagctgctcaacaccaagctggagcagtgggccgaagaggccgtcgcccgtggcggattccacgccaccaccgccttgctcatccagtacgagaactaccgcgactggattgtcaaccacaacgtcgcgtactcggaactcttcctcgacactgccggagtagccagcttcgatgtgtgggaccttctgcccttcacccgaggatacgttcacatcctcgacaaggacccctaccttcaccacttcgcctacgaccctcagtacttcctcaacgagctggacctgctcggtcaggctgccgctactcaactggcccgcgccatctccaactccggtgccatgcagacctacttcgctggggagactatccccggtgataacctcgcgtatgatgccgatttgagcgcctggactgagtacatcccgtaccacttccgtcctaactaccatggcgtgggtacttgctccatgatgccgaaggagatgggcggtgttgttgataatgctgcccgtgtgtatggtgtgcagggactgcgtgtcattgatggttctattcctcctacgcaaatgtcgtcccatgtcatgacggtgttctatgccatggcgctaaaaatttcggatgctatcttggaagattatgcttccatgcagtga

SEQ ID NO: 8 - DNA, 1584 bp, synthetic construct
  source 1..1584: mol_type = other DNA
atggctgacagccgggatcccgccagcgaccagatgcagcactggaaggagcagcgggccgcgcagaaagctgatgtcctgaccactggagctggtaacccagtaggagacaaacttaatgttattacagtagggccccgtgggccccttcttgttcaggatgtggttttcactgatgaaatggctcattttgaccgagagagaattcctgagagagttgtgcatgctaaaggagcaggggcctttggctactttgaggtcacacatgacattaccaaatactccaaggcaaaggtatttgagcatattggaaagaagactcccatcgcagttcggttctccactgttgctggagaatcgggttcagctgacacagttcgggaccctcgtgggtttgcagtgaaattttacacagaagatggtaactgggatctcgttggacaaaacacccccattttcttcatcagggatcccatattgtttccatcttttatccacagccaaaagagaaatcctcagacacatctgaaggatccggacatggtctgggacttctggagcctacgtcctgagtctctgcatcaggtttctttcttgttcagtgatcgggggattccagatggacatcgccacatgaatggatatggatcacatactttcaagctggttaatgcaaatggggaggcagtttattgcaaattccattataagactgaccagggcatcaaacaactttctgttgaagatgcggcgagactttcccaggaagatcctgactatggcatccgggatctttttaacgccattgccacaggaaagtacccctcctggactttttacatccaggtcatgacatttaatcaggcagaaacttttccatttaatccattcgatctcaccaaggtttggcctcacaaggactaccctctcatcccagttggtaaactggtcttaaaccggaatccagttaattactttgctgaggttgaacagatagccttcgacccaagcaacatgccacctggcattgaggccagtcctgacaaaatgcttcagggccgcctttttgcctatcctgacactcaccgccatcgcctgggacccaattatcttcatatacctgtgaactgtccctaccgtgctcgagtggccaactaccagcgtgacggcccgatgtgcatgcaggacaatcagggtggtgctccaaattactaccccaacagctttggtgctccggaacaacagccttctgccctggagcacagcatccaatattctggagaagtgcggagattcaacactgccaatgatgatcaagttactcaggtgcgggcattctatgtgaacgtgctgaatgaggaacagaggaaacgtctgtgtgagaacattgccggccacctgaaggatgcacaaattttcatccagaagaaagcggtcaagcaattcactgaggtccaccctgactacgggagccacatccaggctcttctggacaagtacaatgctgagaagcctaagaatgcgattcacacctttgtgcagtccggatctcacttggcggcaagggagaaggcaaatctgtga

SEQ ID NO: 9 - DNA, 21 bp, synthetic construct
  source 1..21: mol_type = other DNA
atgcagactctccttgtgagc

SEQ ID NO: 10 - DNA, 23 bp, synthetic construct
  source 1..23: mol_type = other DNA
tcactgcatggaagcataatctt

SEQ ID NO: 11 - DNA, 26 bp, synthetic construct
  source 1..26: mol_type = other DNA
tatccatacgatgttcctgattatgc

SEQ ID NO: 12 - DNA, 33 bp, synthetic construct
  source 1..33: mol_type = other DNA
atactgtttaaattaatctatgctagcttattt

SEQ ID NO: 13 - DNA, 32 bp, synthetic construct
  source 1..32: mol_type = other DNA
gaacccccaatcagtgtgctcgtcatcgaaag

SEQ ID NO: 14 - DNA, 32 bp, synthetic construct
  source 1..32: mol_type = other DNA
acactgattgggggttctccgtcagacgagca

SEQ ID NO: 15 - DNA, 32 bp, synthetic construct
  source 1..32: mol_type = other DNA
taccaaccaacaaaccgcgctgatccgctccg

SEQ ID NO: 16 - DNA, 32 bp, synthetic construct
  source 1..32: mol_type = other DNA
cggtttgttggttggtagcgagctccacggtc

SEQ ID NO: 17 - DNA, 32 bp, synthetic construct
  source 1..32: mol_type = other DNA
ctacttccaagcatcctgccatggtgttaatg

SEQ ID NO: 18 - DNA, 32 bp, synthetic construct
  source 1..32: mol_type = other DNA
aggatgcttggaagtagtggccagcagcgatc

SEQ ID NO: 19 - DNA, 32 bp, synthetic construct
  source 1..32: mol_type = other DNA
tggtgttcaaggtactgtccatgccggacccc

SEQ ID NO: 20 - DNA, 32 bp, synthetic construct
  source 1..32: mol_type = other DNA
cagtaccttgaacaccatggcaggatgcgttg

SEQ ID NO: 21 - DNA, 35 bp, synthetic construct
  source 1..35: mol_type = other DNA
tgctccttagccagcaaggcaccacccctcgtgcc

SEQ ID NO: 22 - DNA, 32 bp, synthetic construct
  source 1..32: mol_type = other DNA
ttgctggctaaggagcaccttaccaacatatt

SEQ ID NO: 23 - DNA, 33 bp, synthetic construct
  source 1..33: mol_type = other DNA
caccttccaagagacctttggtgactattccga

SEQ ID NO: 24 - DNA, 32 bp, synthetic construct
  source 1..32: mol_type = other DNA
aggtctcttggaaggtggcgaaccaagcggcc

SEQ ID NO: 25 - DNA, 32 bp, synthetic construct
  source 1..32: mol_type = other DNA
attccaccaaaccaccgccttgctcatccagt

SEQ ID NO: 26 - DNA, 32 bp, synthetic construct
  source 1..32: mol_type = other DNA
cggtggtttggtggaatccgccacgggcgacg

SEQ ID NO: 27 - DNA, 32 bp, synthetic construct
  source 1..32: mol_type = other DNA
ccgccaaatctccaactccggtgccatgcaga

SEQ ID NO: 28 - DNA, 32 bp, synthetic construct
  source 1..32: mol_type = other DNA
agttggagatttggcgggccagttgagtagcg

SEQ ID NO: 29 - DNA, 33 bp, synthetic construct
  source 1..33: mol_type = other DNA
agaaccccgccatcagtgtgctcgtcatcgaaa

SEQ ID NO: 30 - DNA, 32 bp, synthetic construct
  source 1..32: mol_type = other DNA
actgatggcggggttctccgtcagacgagcag

SEQ ID NO: 31 - DNA, 32 bp, synthetic construct
  source 1..32: mol_type = other DNA
taccaacgcccaaaccgcgctgatccgctccg

SEQ ID NO: 32 - DNA, 32 bp, synthetic construct
  source 1..32: mol_type = other DNA
cggtttgggcgttggtagcgagctccacggtc

SEQ ID NO: 33 - DNA, 32 bp, synthetic construct
  source 1..32: mol_type = other DNA
ctacttcgccgcatcctgccatggtgttaatg

SEQ ID NO: 34 - DNA, 32 bp, synthetic construct
  source 1..32: mol_type = other DNA
aggatgcggcgaagtagtggccagcagcgatc

SEQ ID NO: 35 - DNA, 32 bp, synthetic construct
  source 1..32: mol_type = other DNA
atggtgttgccggtactgtccatgccggaccc

SEQ ID NO: 36 - DNA, 32 bp, synthetic construct
  source 1..32: mol_type = other DNA
agtaccggcaacaccatggcaggatgcgttga

SEQ ID NO: 37 - DNA, 35 bp, synthetic construct
  source 1..35: mol_type = other DNA
tgctccttagccaggccggcaccacccctcgtgcc

SEQ ID NO: 38 - DNA, 32 bp, synthetic construct
  source 1..32: mol_type = other DNA
ggcctggctaaggagcaccttaccaacatatt

SEQ ID NO: 39 - DNA, 32 bp, synthetic construct
  source 1..32: mol_type = other DNA
accttcgccgagacctttggtgactattccga

SEQ ID NO: 40 - DNA, 32 bp, synthetic construct
  source 1..32: mol_type = other DNA
aaggtctcggcgaaggtggcgaaccaagcggc

SEQ ID NO: 41 - DNA, 32 bp, synthetic construct
  source 1..32: mol_type = other DNA
attccacgccaccaccgccttgctcatccagt

SEQ ID NO: 42 - DNA, 32 bp, synthetic construct
  source 1..32: mol_type = other DNA
cggtggtggcgtggaatccgccacgggcgacg

SEQ ID NO: 43 - DNA, 32 bp, synthetic construct
  source 1..32: mol_type = other DNA
ccgcgccatctccaactccggtgccatgcaga

SEQ ID NO: 44 - DNA, 32 bp, synthetic construct
  source 1..32: mol_type = other DNA
agttggagatggcgcgggccagttgagtagcg

SEQ ID NO: 45 - DNA, 20 bp, synthetic construct
  source 1..20: mol_type = other DNA
atggctgacagccgggatcc

SEQ ID NO: 46 - DNA, 20 bp, synthetic construct
  source 1..20: mol_type = other DNA
tcacagatttgccttctccc

SEQ ID NO: 47 - DNA, 26 bp, synthetic construct
  source 1..26: mol_type = other DNA
tatccatacgatgttcctgattatgc

SEQ ID NO: 48 - DNA, 33 bp, synthetic construct; identical to SEQ ID NO: 12
  source 1..33: mol_type = other DNA

SEQ ID NO: 49 - DNA, 32 bp, synthetic construct
  source 1..32: mol_type = other DNA
cgttggacaaaacacccccattttcttcatca

SEQ ID NO: 50 - DNA, 32 bp, synthetic construct
  source 1..32: mol_type = other DNA
gggtgttttgtccaacgagatcccagttacca

SEQ ID NO: 51 - DNA, 36 bp, synthetic construct
  source 1..36: mol_type = other DNA
cagggcatcaaacaactttctgttgaagatgcggcg

SEQ ID NO: 52 - DNA, 32 bp, synthetic construct
  source 1..32: mol_type = other DNA
agttgtttgatgccctggtcagtcttataatg

SEQ ID NO: 53 - DNA, 32 bp, synthetic construct
  source 1..32: mol_type = other DNA
tcaagttactcaggtgcgggcattctatgtga

SEQ ID NO: 54 - DNA, 40 bp, synthetic construct
  source 1..40: mol_type = other DNA
gcacctgagtaacttgatcatcattggcagtgttgaatct

SEQ ID NO: 55 - DNA, 32 bp, synthetic construct
  source 1..32: mol_type = other DNA
ggtcaagcaattcactgaggtccaccctgact

SEQ ID NO: 56 - DNA, 32 bp, synthetic construct
  source 1..32: mol_type = other DNA
cagtgaattgcttgaccgctttcttctggatg

SEQ ID NO: 57 - DNA, 32 bp, synthetic construct; identical to SEQ ID NO: 13
  source 1..32: mol_type = other DNA

SEQ ID NO: 58 - DNA, 32 bp, synthetic construct; identical to SEQ ID NO: 14
  source 1..32: mol_type = other DNA

SEQ ID NO: 59 - DNA, 32 bp, synthetic construct
  source 1..32: mol_type = other DNA
gagcaatgccattgaagccagcctcctgactg

SEQ ID NO: 60 - DNA, 33 bp, synthetic construct
  source 1..33: mol_type = other DNA
cttcaatggcattgctcctgatgtagtgtggca

SEQ ID NO: 61 - DNA, 32 bp, synthetic construct
  source 1..32: mol_type = other DNA
gacagagcccctatcattgaggacctgaacgc

SEQ ID NO: 62 - DNA, 32 bp, synthetic construct
  source 1..32: mol_type = other DNA
atgataggggctctgtccgactcgtaggagcc

SEQ ID NO: 63 - DNA, 36 bp, synthetic construct
  source 1..36: mol_type = other DNA
tgatccgctccgccaatggtctcggtggctctactc

SEQ ID NO: 64 - DNA, 32 bp, synthetic construct
  source 1..32: mol_type = other DNA
attggcggagcggatcagcgcggtttgattgt

SEQ ID NO: 65 - DNA, 32 bp, synthetic construct
  source 1..32: mol_type = other DNA
aaatgaggcctggaactgggacaatgtggccg

SEQ ID NO: 66 - DNA, 34 bp, synthetic construct
  source 1..34: mol_type = other DNA
agttccaggcctcatttccaaagacagtctccca

SEQ ID NO: 67 - DNA, 32 bp, synthetic construct
  source 1..32: mol_type = other DNA
tgttaatgccactgtccatgccggaccccgcg

SEQ ID NO: 68 - DNA, 32 bp, synthetic construct
  source 1..32: mol_type = other DNA
ggacagtggcattaacaccatggcaggatgcg

SEQ ID NO: 69 - DNA, 32 bp, synthetic construct
  source 1..32: mol_type = other DNA
atatgttgccaaggtgctccttagccagaacg

SEQ ID NO: 70 - DNA, 33 bp, synthetic construct
  source 1..33: mol_type = other DNA
gcaccttggcaacatattggtcttcgtgcaagg

SEQ ID NO: 71 - DNA, 32 bp, synthetic construct
  source 1..32: mol_type = other DNA
gtcgccttgaacctgcaggaccagaccaccgc

SEQ ID NO: 72 - DNA, 33 bp, synthetic construct
  source 1..33: mol_type = other DNA
tgcaggttcaaggcgacgggcaggtcaacgacg

SEQ ID NO: 73 - DNA, 35 bp, synthetic construct
  source 1..35: mol_type = other DNA
taactaccatgccgtgggtacttgctccatgatgc

SEQ ID NO: 74 - DNA, 32 bp, synthetic construct
  source 1..32: mol_type = other DNA
ccacggcatggtagttaggacggaagtggtac

SEQ ID NO: 75 - DNA, 32 bp, synthetic construct; identical to SEQ ID NO: 49
  source 1..32: mol_type = other DNA

SEQ ID NO: 76 - DNA, 32 bp, synthetic construct; identical to SEQ ID NO: 50
  source 1..32: mol_type = other DNA

SEQ ID NO: 77 - DNA, 32 bp, synthetic construct
  source 1..32: mol_type = other DNA
tgcatgctaaagccgcaggggcctttggctac

SEQ ID NO: 78 - DNA, 32 bp, synthetic construct
  source 1..32: mol_type = other DNA
tgcggctttagcatgcacaactctctcaggaa

SEQ ID NO: 79 - DNA, 32 bp, synthetic construct
  source 1..32: mol_type = other DNA
atcgggccattccagatggacatcgccacatg

SEQ ID NO: 80 - DNA, 36 bp, synthetic construct
  source 1..36: mol_type = other DNA
atctggaatggcccgatcactgaacaagaaagaaac

SEQ ID NO: 81 - DNA, 36 bp, synthetic construct
  source 1..36: mol_type = other DNA
ttgccacagccaagtacccctcctggactttttaca

SEQ ID NO: 82 - DNA, 32 bp, synthetic construct
  source 1..32: mol_type = other DNA
gtacttggctgtggcaatggcgttaaaaagat

SEQ ID NO: 83 - DNA, 32 bp, synthetic construct
  source 1..32: mol_type = other DNA
attgccgcccacctgaaggatgcacaaatttt

SEQ ID NO: 84 - DNA, 34 bp, synthetic construct
  source 1..34: mol_type = other DNA
ttcaggtgggcggcaatgttctcacacagacgtt

SEQ ID NO: 85 - protein, 605 aa, synthetic construct
MQTLLVSSLVVSLAAALPHYIRSNGIEASLLTDPKDVSGRTVDYIIAGGGLTGLTTAARLTENPQISVLVIESGSYESDRGPIIEDLNAYGDIFGSSVDHAYETVELATNNQTALIRSGNGLGGSTLVNGGTWTRPHKAQVDSWETVFGNEGWNWDNVAAYSLQAERARAPNAKQIAAGHYFNASCHGVNGTVHAGPRDTGDDYSPIVKALMSAVEDRGVPTKKDFGCGDPHGVSMFPNTLHEDQVRSDAAREWLLPNYQRPNLQVLTGQYVGKVLLSQNGTTPRAVGVEFGTHKGNTHNVYAKHEVLLAAGSAVSPTILEYSGIGMKSILEPLGIDTVVDLPVGLNLQDQTTATVRSRITSAGAGQGQAAWFATFNETFGDYSEKAHELLNTKLEQWAEEAVARGGFHNTTALLIQYENYRDWIVNHNVAYSELFLDTAGVASFDVWDLLPFTRGYVHILDKDPYLHHFAYDPQYFLNELDLLGQAAATQLARNISNSGAMQTYFAGETIPGDNLAYDADLSAWTEYIPYHFRPNYHGVGTCSMMPKEMGGVVDNAARVYGVQGLRVIDGSIPPTQMSSHVMTVFYAMALKISDAILEDYASMQ

SEQ ID NO: 86 - protein, 580 aa, synthetic construct
MQTLLVSSLVVSLAAALPHYIRSNAIEASLLTDPKDVSGRTVDYIIAGGGLTGLTTAARLTENPNISVLVIESGSYESDRAPIIEDLNAYGDIFGSSVDHAYETVELATNNQTALIRSANGLGGSTLVNGGTWTRPHKAQVDSWETVFGNEAWNWDNVAAYSLQAERARAPNAKQIAAGHYFNASCHGVNATVHAGPRDTGDDYSPIVKALMSAVEDRGVPTKKDFGCGDPHGVSMFPNTLHEDQYVAKVLLSQNGTTPRAVGVEFGTHKGNTHNVYAKHEVLLAAGSAVSPTILEYSGIGMKSILEPLGIDTVVDLPVALNLQDQTTATVRSRITSAGAGQGQAAWFATFNETFGDYSEKAHELLNTKLEQWAEEAVARGGFHNTTALLIQYENYRDWIVNHNVAYSELFLDTAGVASFDVWDLLPFTRGYVHILDKDPYLHHFAYDPQYFLNELDLLGQAAATQLARNISNSGAMQTYFAGETIPGDNLAYDADLSAWTEYIPYHFRPNYHAVGTCSMMPKEMGGVVDNAARVYGVQGLRVIDGSIPPTQMSSHVMTVFYAMALKISDAILEDYASMQ

SEQ ID NO: 87 - protein, 527 aa, synthetic construct
MADSRDPASDQMQHWKEQRAAQKADVLTTGAGNPVGDKLNVITVGPRGPLLVQDVVFTDEMAHFDRERIPERVVHAKGAGAFGYFEVTHDITKYSKAKVFEHIGKKTPIAVRFSTVAGESGSADTVRDPRGFAVKFYTEDGNWDLVGQNTPIFFIRDPILFPSFIHSQKRNPQTHLKDPDMVWDFWSLRPESLHQVSFLFSDRGIPDGHRHMNGYGSHTFKLVNANGEAVYCKFHYKTDQGIKNLSVEDAARLSQEDPDYGIRDLFNAIATGKYPSWTFYIQVMTFNQAETFPFNPFDLTKVWPHKDYPLIPVGKLVLNRNPVNYFAEVEQIAFDPSNMPPGIEASPDKMLQGRLFAYPDTHRHRLGPNYLHIPVNCPYRARVANYQRDGPMCMQDNQGGAPNYYPNSFGAPEQQPSALEHSIQYSGEVRRFNTANDDNVTQVRAFYVNVLNEEQRKRLCENIAGHLKDAQIFIQKKAVKNFTEVHPDYGSHIQALLDKYNAEKPKNAIHTFVQSGSHLAAREKANL

SEQ ID NO: 88 - protein, 527 aa, synthetic construct
MADSRDPASDQMQHWKEQRAAQKADVLTTGAGNPVGDKLNVITVGPRGPLLVQDVVFTDEMAHFDRERIPERVVHAKAAGAFGYFEVTHDITKYSKAKVFEHIGKKTPIAVRFSTVAGESGSADTVRDPRGFAVKFYTEDGNWDLVGNNTPIFFIRDPILFPSFIHSQKRNPQTHLKDPDMVWDFWSLRPESLHQVSFLFSDRAIPDGHRHMNGYGSHTFKLVNANGEAVYCKFHYKTDQGIKNLSVEDAARLSQEDPDYGIRDLFNAIATAKYPSWTFYIQVMTFNQAETFPFNPFDLTKVWPHKDYPLIPVGKLVLNRNPVNYFAEVEQIAFDPSNMPPGIEASPDKMLQGRLFAYPDTHRHRLGPNYLHIPVNCPYRARVANYQRDGPMCMQDNQGGAPNYYPNSFGAPEQQPSALEHSIQYSGEVRRFNTANDDNVTQVRAFYVNVLNEEQRKRLCENIAAHLKDAQIFIQKKAVKNFTEVHPDYGSHIQALLDKYNAEKPKNAIHTFVQSGSHLAAREKANL